European Patent Application EP 4 327 818 A2, published February 28, 2024. Title: Improved anti-senescence compounds and uses for the treatment of cancer. Applicant: Cleara Biotech B.V. Application EP. The sequence listing filed with the application follows.

SEQUENCE LISTING (68 sequences)

SEQ ID NO: 1 - skipped

SEQ ID NO: 2 - protein, 32 aa, Homo sapiens
  SITE 1: note = misc_feature - Xaa can be Leu Thr Leu
  SITE 2: note = misc_feature - Xaa can be Arg or Ser
  SITE 4: note = misc_feature - Xaa can be Lys, Glu, Arg, and His
  SITE 5: note = misc_feature - Xaa can be Ala or Pro
  SITE 6: note = misc_feature - Xaa can be Ala or Ser
  SITE 7: note = misc_feature - Xaa can be Ala or Ser or Fmoc-L-2-(4'-pentenyl)alanine (staple)
  SITE 8: note = misc_feature - Xaa can be Lys, Glu, Arg, or His
  SITE 9: note = misc_feature - Xaa can be Ile or Leu or cyclo-hexyl-alanine
  SITE 10: note = misc_feature - Xaa can be Ala, Gly, Ser, Glu, or Asp
  SITE 11: note = misc_feature - Xaa can be Gly, Gln, Ala, Ser, or Pro or Fmoc-L-2-(4'-pentenyl)alanine (staple)
  SITE 12: note = misc_feature - Xaa can be Ala, Gly, Ser, Glu, or Asp
  REGION 13..14: note = misc_feature - Xaa can be Ile or Leu or cyclo-hexyl-alanine
  SITE 15: note = misc_feature - Xaa can be Glu or Asp
  SITE 17: note = misc_feature - Xaa can be Trp, Tyr, and Phe
  SITE 18: note = misc_feature - Xaa can be Ala or Ser or Fmoc-L-2-(4'-pentenyl)alanine (staple)
  SITE 21: note = misc_feature - Xaa can be Ala or Gly
  SITE 22: note = misc_feature - Xaa can be Trp, Tyr, and Phe
  REGION 23..24: note = misc_feature - Xaa can be Ala
  SITE 25: note = misc_feature - Xaa can be Arg or Lys
  SITE 26: note = misc_feature - Xaa can be Arg
  SITE 28: note = misc_feature - Xaa can be Gly or Ser
  SITE 29: note = misc_feature - Xaa can be Ala or Cys
  REGION 30..31: note = misc_feature - Xaa can be Arg or Lys
  SITE 32: note = misc_feature - Xaa can be Ala or Cys
XXKXXXXXXXXXXXXAXXQNXXXXXXSXXXXX

SEQ ID NO: 3 - skipped

SEQ ID NO: 4 - protein, 14 aa, Homo sapiens
  SITE 2: note = misc_feature - Xaa can be Ala, Gly, Ser, Glu, or Asp
  SITE 3: note = misc_feature - Xaa can be Gly, Gln, Ala, Ser, or Pro
  SITE 4: note = misc_feature - Xaa can be Ala, Gly, Ser, Glu, or Asp
  SITE 7: note = misc_feature - Xaa can be Glu or Asp
  SITE 10: note = misc_feature - Xaa can be Ala or Ser
  SITE 13: note = misc_feature - Xaa can be Ala or Gly
IXXXILXAFXQNXW

SEQ ID NO: 5 - protein, 34 aa, Homo sapiens
LTLRKEPASEIAQSILEAYSQNGWANRRSGGKRP

SEQ ID NO: 6 - protein, 46 aa, Homo sapiens
LTLRKEPASEIAQSILEAYSQNGWANRRSGGKRPPPRRRQRRKKRG

SEQ ID NO: 7 - protein, 34 aa, Homo sapiens
LTLRKEASSEIAQSILDAYSQNGWANRRSSCKRP

SEQ ID NO: 8 - protein, 34 aa, Homo sapiens
LTLRKKASSKIAQSILDAFSQNGWANRRSSCKRP

SEQ ID NO: 9 - protein, 34 aa, Homo sapiens; identical to SEQ ID NO: 5

SEQ ID NO: 10 - protein, 31 aa, Homo sapiens
RKKASSKIAQSILDAFSQNGWANRRSSCKRP

SEQ ID NO: 11 - protein, 31 aa, Homo sapiens
RKKASSKIAAAILDAFSQNGWANRRSSCKRP

SEQ ID NO: 12 - protein, 31 aa, Homo sapiens
RKKASSKIAAAILDAFSQNAWANRRSSCKRP

SEQ ID NO: 13 - protein, 24 aa, Homo sapiens
RKKASSKIAAAILDAFSQNWRRKR

SEQ ID NO: 14 - protein, 24 aa, Homo sapiens
RKKASSKIEAAILDAFSQNWRRKR

SEQ ID NO: 15 - protein, 24 aa, Homo sapiens
RKKASSKIAAEILDAFSQNWRRKR

SEQ ID NO: 16 - protein, 24 aa, Homo sapiens
RKKASSKIEAEILDAFSQNWRRKR

SEQ ID NO: 17 - protein, 22 aa, Homo sapiens
RKKSKIAAAILDAFSQNWRRKR

SEQ ID NO: 18 - protein, 22 aa, Homo sapiens
RKKSKIEAEILDAFSQNWRRKR

SEQ ID NO: 19 - protein, 19 aa, Homo sapiens
AKIAAAILDAFSQNWRRKR

SEQ ID NO: 20 - protein, 19 aa, Homo sapiens
AKIEAAILDAFSQNWRRKR

SEQ ID NO: 21 - protein, 46 aa, Homo sapiens; identical to SEQ ID NO: 6

SEQ ID NO: 22 - protein, 43 aa, Homo sapiens
RKKASSKIAAAILDAFSQNGWANRRSSCKRPPPRRRQRRKKRG

SEQ ID NO: 23 - protein, 43 aa, Homo sapiens
RKKASSKIAAAILDAFSQNAWANRRSSCKRPPPRRRQRRKKRA

SEQ ID NO: 24 - protein, 36 aa, Homo sapiens
RKKASSKIAAAILDAFSQNWRRKRPPRRRQRRKKRG

SEQ ID NO: 25 - protein, 36 aa, Homo sapiens
RKKASSKIEAAILDAFSQNWRRKRPPRRRQRRKKRG

SEQ ID NO: 26 - protein, 36 aa, Homo sapiens
RKKASSKIAAEILDAFSQNWRRKRPPRRRQRRKKRG

SEQ ID NO: 27 - protein, 36 aa, Homo sapiens
RKKASSKIEAEILDAFSQNWRRKRPPRRRQRRKKRG

SEQ ID NO: 28 - protein, 32 aa, Homo sapiens
RKKSKIAAAILDAFSQNWRRKRRRRQRRKKRG

SEQ ID NO: 29 - protein, 32 aa, Homo sapiens
RKKSKIEAEILDAFSQNWRRKRRRRQRRKKRG

SEQ ID NO: 30 - protein, 29 aa, Homo sapiens
AKIAAAILDAFSQNWRRKRRRRQRRKKRG

SEQ ID NO: 31 - protein, 29 aa, Homo sapiens
AKIEAAILDAFSQNWRRKRRRRQRRKKRG

SEQ ID NO: 32 - protein, 91 aa, Homo sapiens
PRKGGSRRNAWGNQSYAELISQAIESAPEKRLTLAQIYEWMVRTVPYFKDKGDSNSSAGWKNSIRHNLSLHSKFIKVHNEATGKSSWWMLN

SEQ ID NO: 33 - protein, 34 aa, Homo sapiens
PRKGGSRRNAWGNQSYAELISQAIESAPEKRLTL

SEQ ID NO: 34 - protein, 22 aa, Homo sapiens
AMDDLMLSPDDIEQWFTEDPGP

SEQ ID NO: 35 - protein, 10 aa, Homo sapiens
LTLRKEASSE

SEQ ID NO: 36 - skipped

SEQ ID NO: 37 - protein, 6 aa, Homo sapiens
IAQSIL

SEQ ID NO: 38 - protein, 10 aa, Homo sapiens
ANRRSSCKRP

SEQ ID NO: 39 - protein, 505 aa, Homo sapiens
MDPGNENSATEAAAIIDLDPDFEPQSRPRSCTWPLPRPEIANQPSEPPEVEPDLGEKVHTEGRSEPILLPSRLPEPAGGPQPGILGAVTGPRKGGSRRNAWGNQSYAELISQAIESAPEKRLTLAQIYEWMVRTVPYFKDKGDSNSSAGWKNSIRHNLSLHSKFIKVHNEATGKSSWWMLNPEGGKSGKAPRRRAASMDSSSKLLRGRSKAPKKKPSVLPAPPEGATPTSPVGHFAKWSGSPCSRNREEADMWTTFRPRSSSNASSVSTRLSPLRPESEVLAEEIPASVSSYAGGVPPTLNEGLELLDGLNLTSSHSLLSRSGLSGFSLQHPGVTGPLHTYSSSLFSPAEGPLSAGEGCFSSSQALEALLTSDTPPPPADVLMTQVDPILSQAPTLLLLGGLPSSSKLATGVGLCPKPLEAPGPSSLVPTLSMIAPPPVMASAPIPKALGTPVLTPPTEAASQDRMPQDLDLDMYMENLECDMDNIISDLMDEGEGLDFNFEPDP

SEQ ID NO: 40 - protein, 393 aa, Homo sapiens [sequence omitted]

SEQ ID NO: 41 - protein, 12 aa, Homo sapiens
GRKKRRQRRRPP

SEQ ID NO: 42 - protein, 34 aa, Homo sapiens; identical to SEQ ID NO: 33

SEQ ID NO: 43 - protein, 5 aa, Homo sapiens
SQNAW

SEQ ID NO: 44 - protein, 5 aa, Homo sapiens
SQNGW

SEQ ID NO: 45 - protein, 4 aa, Homo sapiens
SQNW

SEQ ID NO: 46 - protein, 5 aa, Homo sapiens
KIAAA

SEQ ID NO: 47 - protein, 5 aa, Homo sapiens
KIEAA

SEQ ID NO: 48 - protein, 5 aa, Homo sapiens
KIAAE

SEQ ID NO: 49 - protein, 5 aa, Homo sapiens
KIEAE

SEQ ID NO: 50 - protein, 4 aa, Homo sapiens
SQNG

SEQ ID NO: 51 - protein, 4 aa, Homo sapiens
AANG

SEQ ID NO: 52 - protein, 4 aa, Homo sapiens
SQAG

SEQ ID NO: 53 - protein, 36 aa, Homo sapiens; identical to SEQ ID NO: 27

SEQ ID NO: 54 - protein, 31 aa, Homo sapiens
RKKSKIEAEILDAFSQNWRKRRRRQRRKKRG

SEQ ID NO: 55 - protein, 28 aa, Homo sapiens
AKIEAAILDAFSQNWRKRRRRQRRKKRG

SEQ ID NO: 56 - protein, 28 aa, Homo sapiens
AKIEAEILDAFSQNWRKRRRRQRRKKRG

SEQ ID NO: 57 - protein, 28 aa, Homo sapiens
AKIEAAILDEFSQNWRKRRRRQRRKKRG

SEQ ID NO: 58 - protein, 36 aa, Homo sapiens
  SITE 6: note = misc_feature - Fmoc-L-2-(4'-pentenyl)alanine
  SITE 10: note = misc_feature - Fmoc-L-2-(4'-pentenyl)alanine
RKKASXKIAXAILDAFSQNWRRKRPPRRRQRRKKRG

SEQ ID NO: 59 - protein, 43 aa, Homo sapiens
  SITE 12: note = misc_feature - cyclo-hexyl-alanine
RKKASSKIAAAXLDAFSQNAWANRRSSCKRPPPRRRQRRKKRA

SEQ ID NO: 60 - protein, 28 aa, Homo sapiens
  SITE 15: note = misc_feature - 2-Me-tryptophane
AKIEAAILDAFSQNXRKRRRRQRRKKRG

SEQ ID NO: 61 - protein, 28 aa, Homo sapiens
  SITE 15: note = misc_feature - 2-Me-tryptophane
AKIEAEILEAFSQNXRKRRRRQRRKKRG

SEQ ID NO: 62 - protein, 28 aa, Homo sapiens
  SITE 7: note = misc_feature - cyclo-hexyl-alanine
  SITE 15: note = misc_feature - 2-Me-tryptophane
AKIEAAXLDAFSQNXRKRRRRQRRKKRG

SEQ ID NO: 63 - protein, 36 aa, Homo sapiens
  SITE 20: note = misc_feature - 2-Me-tryptophane
RKKASSKIEAEILDAFSQNXRRKRPPRRRQRRKKRG

SEQ ID NO: 64 - protein, 36 aa, Homo sapiens
  SITE 12: note = misc_feature - cyclo-hexyl alanine
  SITE 20: note = misc_feature - 2-Me-tryptophane
RKKASSKIEAEXLDAFSQNXRRKRPPRRRQRRKKRG

SEQ ID NO: 65 - protein, 36 aa, Homo sapiens
  SITE 20: note = misc_feature - cyclo-hexyl alanine
  SITE 20: note = misc_feature - 2-Me-tryptophane
RKKASSKIEAEIXDAFSQNXRRKRPPRRRQRRKKRG

SEQ ID NO: 66 - protein, 13 aa, Homo sapiens
ARKKRRQRRRPPP

SEQ ID NO: 67 - protein, 31 aa, Homo sapiens
RKKSKIAAAILDAFSQNWRKRRRRQRRKKRG

SEQ ID NO: 68 - protein, 36 aa, Homo sapiens; identical to SEQ ID NO: 25